European Patent Specification EP 3 746 440 B1, published July 5, 2023. Title: PIPECOLIC ESTERS FOR INHIBITION OF THE PROTEASOME. Applicant: GACZYNSKA, Maria OSMULSKI, Pawel A. GILETTO, Matt. The sequence listing filed with the application follows.

SEQUENCE LISTING (1 sequence)

SEQ ID NO: 1 - protein, 10 aa, Artificial Sequence
  synthetic construct
KNMSIKKLWK